European Patent Specification EP 2 970 477 B1, published October 4, 2023. Title: BISPECIFIC-FC MOLECULES. Applicant: AMGEN INC. Application --to be assigned--. The sequence listing filed with the application follows.

SEQUENCE LISTING (92 sequences)

SEQ ID NO: 1 - protein, 9 aa, Artificial Sequence
  source: /note="Description of Artificial Sequence: Synthetic amino acid sequence immediately preceding HC CDR1"
  MOD_RES (2)..(9): Any amino acid
CXXXXXXXX

SEQ ID NO: 2 - protein, 5 aa, Artificial Sequence
  source: /note="Description of Artificial Sequence: Synthetic amino acid sequence preceding HC CDR2"
LEWIG

SEQ ID NO: 3 - protein, 4 aa, Artificial Sequence
  source: /note="Description of Artificial Sequence: Synthetic amino acid sequence following HC CDR3"
  MOD_RES (3)..(3): Any amino acid
WGXG

SEQ ID NO: 4 - protein, 4 aa, Artificial Sequence
  source: /note="Description of Artificial Sequence: Synthetic amino acid sequence following LC CDR3"
  MOD_RES (3)..(3): Any amino acid
FGXG

SEQ ID NO: 5 - protein, 119 aa, Artificial Sequence
  source: /note="Description of Artificial Sequence: Synthetic amino acid sequence of anti-HER2 VH region"
EVQLLEQSGAELVRPGALVKLSCKASGFKIKDYFVNWVKQRPEQGLEWIGWIDPENDNSLYGPNFQDKASITADTSSNTGYLQLSGLTSEDTAVYYCALYYGSRGDAMDYWGQGTTVTV

SEQ ID NO: 6 - protein, 107 aa, Artificial Sequence
  source: /note="Description of Artificial Sequence: Synthetic amino acid sequence of anti-HER2 VL region"
ELVMTQTPSSLSASLGDRVTISCRASQDISNYLNWYQQKPDGTVKLLIYYTSRLHSGVPSRFSGSGSGTDYSLTISNLEQEDIATYFCQQGNTLPLTFGAGTKLEIK

SEQ ID NO: 7 - protein, 125 aa, Artificial Sequence
  source: /note="Description of Artificial Sequence: Synthetic amino acid sequence of anti-CD3 VH region"
EVQLVESGGGLVQPGGSLKLSCAASGFTFNSYAMNWVRQAPGKGLEWVARIRSKYNNYATYYADSVKGRFTISRDDSKNTAYLQMNNLKTEDTAVYYCVRHGNFGNSYVSWWAYWGQGTLVTVSS

SEQ ID NO: 8 - protein, 109 aa, Artificial Sequence
  source: /note="Description of Artificial Sequence: Synthetic amino acid sequence of anti-CD3 VL region"
QTVVTQEPSLTVSPGGTVTLTCGSSTGAVTSGNYPNWVQQKPGQAPRGLIGGTKFLAPGTPARFSGSLLGGKAALTLSGVQPEDEAEYYCVLWYSNRWVFGGGTKLTVL

SEQ ID NO: 9 - protein, 518 aa, Artificial Sequence
  source: /note="Description of Artificial Sequence: Synthetic amino acid sequence of a single chain anti-HER2/CD3 (P136629.3) P136629.3 aHer2(D3)scFv-aCD3(F12Q)scFv"
EVQLLEQSGAELVRPGALVKLSCKASGFKIKDYFVNWVKQRPEQGLEWIGWIDPENDNSLYGPNFQDKASITADTSSNTGYLQLSGLTSEDTAVYYCALYYGSRGDAMDYWGQGTTVTVSSGGGGSGGGGSGGGGSELVMTQTPSSLSASLGDRVTISCRASQDISNYLNWYQQKPDGTVKLLIYYTSRLHSGVPSRFSGSGSGTDYSLTISNLEQEDIATYFCQQGNTLPLTFGAGTKLEIKSGGGGSEVQLVESGGGLVQPGGSLKLSCAASGFTFNSYAMNWVRQAPGKGLEWVARIRSKYNNYATYYADSVKGRFTISRDDSKNTAYLQMNNLKTEDTAVYYCVRHGNFGNSYVSWWAYWGQGTLVTVSSGGGGSGGGGSGGGGSQTVVTQEPSLTVSPGGTVTLTCGSSTGAVTSGNYPNWVQQKPGQAPRGLIGGTKFLAPGTPARFSGSLLGGKAALTLSGVQPEDEAEYYCVLWYSNRWVFGGGTKLTVLAAADYKDDDDKGSSHHHHHH

SEQ ID NO: 10 - protein, 742 aa, Artificial Sequence
  source: /note="Description of Artificial Sequence: Synthetic amino acid sequence of an anti-HER2/CD3 Bi-Fc (P136632.3) D356K, D399K, L234A, L235A P136632.3 (aHer2(D3)scFv-aCD3 (F12Q)scFv-FcAAKK)"
EVQLLEQSGAELVRPGALVKLSCKASGFKIKDYFVNWVKQRPEQGLEWIGWIDPENDNSLYGPNFQDKASITADTSSNTGYLQLSGLTSEDTAVYYCALYYGSRGDAMDYWGQGTTVTVSSGGGGSGGGGSGGGGSELVMTQTPSSLSASLGDRVTISCRASQDISNYLNWYQQKPDGTVKLLIYYTSRLHSGVPSRFSGSGSGTDYSLTISNLEQEDIATYFCQQGNTLPLTFGAGTKLEIKSGGGGSEVQLVESGGGLVQPGGSLKLSCAASGFTFNSYAMNWVRQAPGKGLEWVARIRSKYNNYATYYADSVKGRFTISRDDSKNTAYLQMNNLKTEDTAVYYCVRHGNFGNSYVSWWAYWGQGTLVTVSSGGGGSGGGGSGGGGSQTVVTQEPSLTVSPGGTVTLTCGSSTGAVTSGNYPNWVQQKPGQAPRGLIGGTKFLAPGTPARFSGSLLGGKAALTLSGVQPEDEAEYYCVLWYSNRWVFGGGTKLTVLAAAEPKSSDKTHTCPPCPAPEAAGGPSVFLFPPKPKDTLMISRTPEVTCVVVDVSHEDPEVKFNWYVDGVEVHNAKTKPREEQYNSTYRVVSVLTVLHQDWLNGKEYKCKVSNKALPAPIEKTISKAKGQPREPQVYTLPPSRKEMTKNQVSLTCLVKGFYPSDIAVEWESNGQPENNYKTTPPVLKSDGSFFLYSKLTVDKSRWQQGNVFSCSVMHEALHNHYTQKSLSLSPGKAAAHHHHHH

SEQ ID NO: 11 - DNA, 2226 bp, Artificial Sequence
  source: /note="Description of Artificial Sequence: Synthetic nucleic acid sequence encoding SEQ ID NO:10 aHer2(D3) scFv-aCD3(F12Q)scFv-FcAAKK)"
gaggtgcagctgctcgagcagtctggagctgagcttgtgaggccaggggccttagtcaagttgtcctgcaaagcttctggcttcaaaattaaagactactttgtgaactgggtgaagcagaggcctgaacagggcctggagtggattggatggattgatcctgagaatgataatagtttatatggcccgaacttccaggacaaggccagtatcacagcagacacatcctccaacacaggctacctgcagctcagcggcctgacatctgaggacactgccgtctattactgtgctctttattacggaagtaggggggatgctatggactactggggccaagggaccacggtcaccgtctcctcaggtggtggtggttctggcggcggcggctccggtggtggtggttctgagctcgtgatgacccagactccatcctccctgtctgcctctctgggagacagagtcaccatcagttgcagggcaagtcaggacattagcaattatttaaactggtatcagcagaaaccagatggaactgttaaactcctgatctactacacatcaagattacactcaggagtcccatcaaggttcagtggcagtgggtctggaacagattattctctcaccattagcaacctggagcaagaagatattgccacttacttttgccaacagggtaatacgcttccgctcacgttcggtgctgggaccaagcttgagatcaaatccggaggtggtggatccgaggtgcagctggtcgagtctggaggaggattggtgcagcctggagggtcattgaaactctcatgtgcagcctctggattcaccttcaatagctacgccatgaactgggtccgccaggctccaggaaagggtttggaatgggttgctcgcataagaagtaaatataataattatgcaacatattatgccgattcagtgaaaggcaggttcaccatctccagagatgattcaaaaaacactgcctatctacaaatgaacaacttgaaaactgaggacactgccgtgtactactgtgtgagacatgggaacttcggtaatagctacgtttcctggtgggcttactggggccaagggactctggtcaccgtctcctcaggtggtggtggttctggcggcggcggctccggtggtggtggttctcagactgttgtgactcaggaaccttcactcaccgtatcacctggtggaacagtcacactcacttgtggctcctcgactggggctgttacatctggcaactacccaaactgggtccaacaaaaaccaggtcaggcaccccgtggtctaataggtgggactaagttcctcgcccccggtactcctgccagattctcaggctccctgcttggaggcaaggctgccctcaccctctcaggggtacagccagaggatgaggcagaatattactgtgttctatggtacagcaaccgctgggtgttcggtggaggaaccaaactgactgtcctagcggccgcagagcccaaatcttctgacaaaactcacacatgccccccgtgcccagcacctgaagcagctgggggaccgtcagtcttcctcttccccccaaaacccaaggacaccctcatgatctcccggacccctgaggtcacatgcgtggtggtggacgtgagccacgaagaccctgaggtcaagttcaactggtacgtggacggcgtggaggtgcataatgccaagacaaagccgcgagaggagcagtacaacagcacgtaccgtgtggtcagcgtcctcaccgtcctgcaccaggactggctgaatggcaaggagtacaagtgcaaggtctccaacaaagccctcccagcccccatcgagaaaaccatctccaaagccaaagggcagccccgagaaccacaggtgtacaccctgcccccatcccggaaggagatgaccaagaaccaggtcagcctgacctgcctggtcaaaggcttctatcccagcgacatcgccgtggagtgggagagcaatgggcagccggagaacaactacaagaccacgcctcccgtgctgaagtccgacggctccttcttcctctatagcaagctcaccgtggacaagagcaggtggcagcaggggaacgtcttctcatgctccgtgatgcatgaggctctgcacaaccactacacgcagaagagcctctccctgtctccgggtaaagctgcagcgcatcaccaccaccatcac

SEQ ID NO: 12 - protein, 243 aa, Artificial Sequence
  source: /note="Description of Artificial Sequence: Synthetic amino acid sequence encoding a human IgG1 Fc polypeptide containing alterations K392D and K409D, plus L234A and L235A"
HMSSVSAQAAAEPKSSDKTHTCPPCPAPEAAGGPSVFLFPPKPKDTLMISRTPEVTCVVVDVSHEDPEVKFNWYVDGVEVHNAKTKPREEQYNSTYRVVSVLTVLHQDWLNGKEYKCKVSNKALPAPIEKTISKAKGQPREPQVYTLPPSREEMTKNQVSLTCLVKGFYPSDIAVEWESNGQPENNYDTTPPVLDSDGSFFLYSDLTVDKSRWQQGNVFSCSVMHEALHNHYTQKSLSLSPGK

SEQ ID NO: 13 - DNA, 729 bp, Artificial Sequence
  source: /note="Description of Artificial Sequence: Synthetic nucleic acid sequence encoding SEQ ID NO:12"
cacatgtcttcggtaagtgcacaggcggccgcagagcccaaatcttctgacaaaactcacacatgcccaccgtgcccagcacctgaagcagctgggggaccgtcagtcttcctcttccccccaaaacccaaggacaccctcatgatctcccggacccctgaggtcacatgcgtggtggtggacgtgagccacgaagaccctgaggtcaagttcaactggtacgtggacggcgtggaggtgcataatgccaagacaaagccgcgggaggagcagtacaacagcacgtaccgtgtggtcagcgtcctcaccgtcctgcaccaggactggctgaatggcaaggagtacaagtgcaaggtctccaacaaagccctcccagcccccatcgagaaaaccatctccaaagccaaagggcagccccgagaaccacaggtgtacaccctgcccccatcccgggaggagatgaccaagaaccaggtcagcctgacctgcctggtcaaaggcttctatcccagcgacatcgccgtggagtgggagagcaatgggcagccggagaacaactacgacaccacgcctcccgtgctggactccgacggctccttcttcctctatagcgacctcaccgtggacaagagcaggtggcagcaggggaacgtcttctcatgctccgtgatgcatgaggctctgcacaaccactacacgcagaagagcctctccctgtctccgggtaaa

SEQ ID NO: 14 - protein, 518 aa, Artificial Sequence
  source: /note="Description of Artificial Sequence: Synthetic amino acid sequence of a single chain anti-FOLR1/CD3 molecule P136637.3 aFOLR1(5G1)scFv-aCD3(F12Q)scFv"
QVQLQESGPGLVKPSQTLSLTCTVSGGSISSGAYYWTWIRQHPGKGLEWIGYIYYSGSTYYNPSLKSRVSISIDTSKNQFSLKLSSVTAADTAVYYCARGSSSWFDYWGQGTLVTVSSGGGGSGGGGSGGGGSQSVLTQPPSVSEAPRQRVTISCSGSSSNIGNNAVNWYQQLPGKAPKLLIYYDDMLSSGVSDRFSGSKSGTSASLAISGLQSEDEADYYCAAWDDSLNGVVFGGGTKLTVLSGGGGSEVQLVESGGGLVQPGGSLKLSCAASGFTFNSYAMNWVRQAPGKGLEWVARIRSKYNNYATYYADSVKGRFTISRDDSKNTAYLQMNNLKTEDTAVYYCVRHGNFGNSYVSWWAYWGQGTLVTVSSGGGGSGGGGSGGGGSQTVVTQEPSLTVSPGGTVTLTCGSSTGAVTSGNYPNWVQQKPGQAPRGLIGGTKFLAPGTPARFSGSLLGGKAALTLSGVQPEDEAEYYCVLWYSNRWVFGGGTKLTVLAAADYKDDDDKGSSHHHHHH

SEQ ID NO: 15 - protein, 742 aa, Artificial Sequence
  source: /note="Description of Artificial Sequence: Synthetic amino acid sequence of an anti-FOLR1/CD3 Bi-Fc P136635.4 (aFOLR1(5G1)scFv-aCD3(F12Q)scFv-FcAAKK)"
QVQLQESGPGLVKPSQTLSLTCTVSGGSISSGAYYWTWIRQHPGKGLEWIGYIYYSGSTYYNPSLKSRVSISIDTSKNQFSLKLSSVTAADTAVYYCARGSSSWFDYWGQGTLVTVSSGGGGSGGGGSGGGGSQSVLTQPPSVSEAPRQRVTISCSGSSSNIGNNAVNWYQQLPGKAPKLLIYYDDMLSSGVSDRFSGSKSGTSASLAISGLQSEDEADYYCAAWDDSLNGVVFGGGTKLTVLSGGGGSEVQLVESGGGLVQPGGSLKLSCAASGFTFNSYAMNWVRQAPGKGLEWVARIRSKYNNYATYYADSVKGRFTISRDDSKNTAYLQMNNLKTEDTAVYYCVRHGNFGNSYVSWWAYWGQGTLVTVSSGGGGSGGGGSGGGGSQTVVTQEPSLTVSPGGTVTLTCGSSTGAVTSGNYPNWVQQKPGQAPRGLIGGTKFLAPGTPARFSGSLLGGKAALTLSGVQPEDEAEYYCVLWYSNRWVFGGGTKLTVLAAAEPKSSDKTHTCPPCPAPEAAGGPSVFLFPPKPKDTLMISRTPEVTCVVVDVSHEDPEVKFNWYVDGVEVHNAKTKPREEQYNSTYRVVSVLTVLHQDWLNGKEYKCKVSNKALPAPIEKTISKAKGQPREPQVYTLPPSRKEMTKNQVSLTCLVKGFYPSDIAVEWESNGQPENNYKTTPPVLKSDGSFFLYSKLTVDKSRWQQGNVFSCSVMHEALHNHYTQKSLSLSPGKAAAHHHHHH

SEQ ID NO: 16 - DNA, 2226 bp, Artificial Sequence
  source: /note="Description of Artificial Sequence: Synthetic nucleic acid sequence encoding SEQ ID NO:15 (aFOLR1(5G1) scFv-aCD3(F12Q)scFv-FcAAKK)"
caggtgcagctgcaggagtcgggcccaggactggtgaagccttcacagaccctgtccctcacctgcactgtctctggtggctccatcagcagtggtgcttactactggacctggatccgccagcacccagggaagggcctggagtggattgggtacatctattacagtgggagcacctactacaacccgtccctcaagagtcgagttagcatatcaatagacacgtctaagaaccagttctccctgaagctgagctctgtgactgccgcggacacggccgtgtattactgtgcgcgaggcagcagcagctggttcgactactggggccagggaaccctggtcaccgtctcctcaggaggcggcggttcaggcggaggtggctctggcggtggcggaagtcagtctgtgctgactcagccaccctcggtgtctgaagcccccaggcagagggtcaccatctcctgttctggaagcagctccaacatcggaaataatgctgtaaactggtaccagcagctcccaggaaaggctcccaaactcctcatctattatgatgatatgttgtcttcaggggtctcggaccgattttctggctccaagtctggcacctcagcctccctggccatcagtgggctccagtctgaggatgaggctgattattactgtgcagcatgggatgacagcctgaatggtgtggtattcggcggagggaccaagctgaccgtcctatccggaggtggtggatccgaggtgcagctggtcgagtctggaggaggattggtgcagcctggagggtcattgaaactctcatgtgcagcctctggattcaccttcaatagctacgccatgaactgggtccgccaggctccaggaaagggtttggaatgggttgctcgcataagaagtaaatataataattatgcaacatattatgccgattcagtgaaaggcaggttcaccatctccagagatgattcaaaaaacactgcctatctacaaatgaacaacttgaaaactgaggacactgccgtgtactactgtgtgagacatgggaacttcggtaatagctacgtttcctggtgggcttactggggccaagggactctggtcaccgtctcctcaggtggtggtggttctggcggcggcggctccggtggtggtggttctcagactgttgtgactcaggaaccttcactcaccgtatcacctggtggaacagtcacactcacttgtggctcctcgactggggctgttacatctggcaactacccaaactgggtccaacaaaaaccaggtcaggcaccccgtggtctaataggtgggactaagttcctcgcccccggtactcctgccagattctcaggctccctgcttggaggcaaggctgccctcaccctctcaggggtacagccagaggatgaggcagaatattactgtgttctatggtacagcaaccgctgggtgttcggtggaggaaccaaactgactgtcctagcggccgcagagcccaaatcttctgacaaaactcacacatgccccccgtgcccagcacctgaagcagctgggggaccgtcagtcttcctcttccccccaaaacccaaggacaccctcatgatctcccggacccctgaggtcacatgcgtggtggtggacgtgagccacgaagaccctgaggtcaagttcaactggtacgtggacggcgtggaggtgcataatgccaagacaaagccgcgagaggagcagtacaacagcacgtaccgtgtggtcagcgtcctcaccgtcctgcaccaggactggctgaatggcaaggagtacaagtgcaaggtctccaacaaagccctcccagcccccatcgagaaaaccatctccaaagccaaagggcagccccgagaaccacaggtgtacaccctgcccccatcccggaaggagatgaccaagaaccaggtcagcctgacctgcctggtcaaaggcttctatcccagcgacatcgccgtggagtgggagagcaatgggcagccggagaacaactacaagaccacgcctcccgtgctgaagtccgacggctccttcttcctctatagcaagctcaccgtggacaagagcaggtggcagcaggggaacgtcttctcatgctccgtgatgcatgaggctctgcacaaccactacacgcagaagagcctctccctgtctccgggtaaagctgcagcgcatcaccaccaccatcac

SEQ ID NO: 17 - protein, 5 aa, Artificial Sequence
  source: /note="Description of Artificial Sequence: Synthetic linker peptide"
TVAAP

SEQ ID NO: 18 - protein, 6 aa, Artificial Sequence
  source: /note="Description of Artificial Sequence: Synthetic linker peptide"
ASTKGP

SEQ ID NO: 19 - protein, 10 aa, Artificial Sequence
  source: /note="Description of Artificial Sequence: Synthetic linker peptide"
GGGGSGGGGS

SEQ ID NO: 20 - protein, 8 aa, Artificial Sequence
  source: /note="Description of Artificial Sequence: Synthetic linker peptide"
GGGGSAAA

SEQ ID NO: 21 - protein, 15 aa, Artificial Sequence
  source: /note="Description of Artificial Sequence: Synthetic linker peptide"
GGGGSGGGGSGGGGS

SEQ ID NO: 22 - protein, 186 aa, Homo sapiens
  source: /note="Mature amino acid sequence of CD3 epsilon chain of Homo sapiens"
QDGNEEMGGITQTPYKVSISGTTVILTCPQYPGSEILWQHNDKNIGGDEDDKNIGSDEDHLSLKEFSELEQSGYYVCYPRGSKPEDANFYLYLRARVCENCMEMDVMSVATIVIVDICITGGLLLLVYYWSKNRKAKAKPVTRGAGAGGRQRGQNKERPPPVPNPDYEPIRKGQRDLYSGLNQRRI

SEQ ID NO: 23 - protein, 177 aa, Macaca fascicularis
  source: /note="Mature amino acid sequence of CD3 epsilon chain of Macaca fascicularis"
QDGNEEMGSITQTPYQVSISGTTVILTCSQHLGSEAQWQHNGKNKGDSGDQLFLPEFSEMEQSGYYVCYPRGSNPEDASHHLYLKARVCENCMEMDVMAVATIVIVDICITLGLLLLVYYWSKNRKAKAKPVTRGAGAGGRQRGQNKERPPPVPNPDYEPIRKGQQDLYSGLNQRRI

SEQ ID NO: 24 - protein, 5 aa, Artificial Sequence
  source: /note="Description of Artificial Sequence: Synthetic peptide which is a portion of an epitope of CD3 epsilon"
QDGNE

SEQ ID NO: 25 - protein, 232 aa, Homo sapiens
  source: /note="amino acid sequence of human IgG1 Fc region"
EPKSCDKTHTCPPCPAPELLGGPSVFLFPPKPKDTLMISRTPEVTCVVVDVSHEDPEVKFNWYVDGVEVHNAKTKPREEQYNSTYRVVSVLTVLHQDWLNGKEYKCKVSNKALPAPIEKTISKAKGQPREPQVYTLPPSRDELTKNQVSLTCLVKGFYPSDIAVEWESNGQPENNYKTTPPVLDSDGSFFLYSKLTVDKSRWQQGNVFSCSVMHEALHNHYTQKSLSLSPGK

SEQ ID NO: 26 - protein, 228 aa, Homo sapiens
  source: /note="amino acid sequence of human IgG2 Fc region"
ERKCCVECPPCPAPPVAGPSVFLFPPKPKDTLMISRTPEVTCVVVDVSHEDPEVQFNWYVDGMEVHNAKTKPREEQFNSTFRVVSVLTVVHQDWLNGKEYKCKVSNKGLPAPIEKTISKTKGQPREPQVYTLPPSREEMTKNQVSLTCLVKGFYPSDIAVEWESNGQPENNYKTTPPMLDSDGSFFLYSKLTVDKSRWQQGNVFSCSVMHEALHNHYTQKSLSLSPGK

SEQ ID NO: 27 - protein, 279 aa, Homo sapiens
  source: /note="amino acid sequence of human IgG3 Fc region"
ELKTPLGDTTHTCPRCPEPKSCDTPPPCPRCPEPKSCDTPPPCPRCPEPKSCDTPPPCPRCPAPELLGGPSVFLFPPKPKDTLMISRTPEVTCVVVDVSHEDPEVQFKWYVDGVEVHNAKTKPREEQYNSTFRVVSVLTVLHQDWLNGKEYKCKVSNKALPAPIEKTISKTKGQPREPQVYTLPPSREEMTKNQVSLTCLVKGFYPSDIAVEWESSGQPENNYNTTPPMLDSDGSFFLYSKLTVDKSRWQQGNIFSCSVMHEALHNRFTQKSLSLSPGK

SEQ ID NO: 28 - protein, 229 aa, Homo sapiens
  source: /note="amino acid sequence of human IgG4 Fc region"
ESKYGPPCPSCPAPEFLGGPSVFLFPPKPKDTLMISRTPEVTCVVVDVSQEDPEVQFNWYVDGVEVHNAKTKPREEQFNSTYRVVSVLTVLHQDWLNGKEYKCKVSNKGLPSSIEKTISKAKGQPREPQVYTLPPSQEEMTKNQVSLTCLVKGFYPSDIAVEWESNGQPENNYKTTPPVLDSDGSFFLYSRLTVDKSRWQEGNVFSCSVMHEALHNHYTQKSLSLSLGK

SEQ ID NO: 29 - protein, 125 aa, Artificial Sequence
  source: /note="Description of Artificial Sequence: Synthetic amino acid sequence of an anti-CD3-epsilon VH region (12C)"
EVQLVESGGGLVQPGGSLKLSCAASGFTFNKYAMNWVRQAPGKGLEWVARIRSKYNNYATYYADSVKDRFTISRDDSKNTAYLQMNNLKTEDTAVYYCVRHGNFGNSYISYWAYWGQGTLVTVSS

SEQ ID NO: 30 - DNA, 375 bp, Artificial Sequence
  source: /note="Description of Artificial Sequence: Synthetic nucleic acid sequence encoding SEQ ID NO:29"
gaggtgcagctggtcgagtctggaggaggattggtgcagcctggagggtcattgaaactctcatgtgcagcctctggattcaccttcaataagtacgccatgaactgggtccgccaggctccaggaaagggtttggaatgggttgctcgcataagaagtaaatataataattatgcaacatattatgccgattcagtgaaagacaggttcaccatctccagagatgattcaaaaaacactgcctatctacaaatgaacaacttgaaaactgaggacactgccgtgtactactgtgtgagacatgggaacttcggtaatagctacatatcctactgggcttactggggccaagggactctggtcaccgtctcctca

SEQ ID NO: 31 - protein, 109 aa, Artificial Sequence; identical to SEQ ID NO: 8
  source: /note="Description of Artificial Sequence: Synthetic amino acid sequence of an anti-CD3-epsilon VL region (12C)"

SEQ ID NO: 32 - DNA, 327 bp, Artificial Sequence
  source: /note="Description of Artificial Sequence: Synthetic nucleic acid sequence encoding SEQ ID NO:31"
cagactgttgtgactcaggaaccttcactcaccgtatcacctggtggaacagtcacactcacttgtggctcctcgactggggctgttacatctggcaactacccaaactgggtccaacaaaaaccaggtcaggcaccccgtggtctaataggtgggactaagttcctcgcccccggtactcctgccagattctcaggctccctgcttggaggcaaggctgccctcaccctctcaggggtacagccagaggatgaggcagaatattactgtgttctatggtacagcaaccgctgggtgttcggtggaggaaccaaactgactgtccta

SEQ ID NO: 33 - protein, 511 aa, Artificial Sequence
  source: /note="Description of Artificial Sequence: Synthetic amino acid sequence of an anti-CD33/CD3 bispecific single chain molecule"
QVQLVQSGAEVKKPGESVKVSCKASGYTFTNYGMNWVKQAPGQGLEWMGWINTYTGEPTYADKFQGRVTMTTDTSTSTAYMEIRNLGGDDTAVYYCARWSWSDGYYVYFDYWGQGTSVTVSSGGGGSGGGGSGGGGSDIVMTQSPDSLTVSLGERTTINCKSSQSVLDSSTNKNSLAWYQQKPGQPPKLLLSWASTRESGIPDRFSGSGSGTDFTLTIDSPQPEDSATYYCQQSAHFPITFGQGTRLEIKSGGGGSEVQLVESGGGLVQPGGSLKLSCAASGFTFNKYAMNWVRQAPGKGLEWVARIRSKYNNYATYYADSVKDRFTISRDDSKNTAYLQMNNLKTEDTAVYYCVRHGNFGNSYISYWAYWGQGTLVTVSSGGGGSGGGGSGGGGSQTVVTQEPSLTVSPGGTVTLTCGSSTGAVTSGNYPNWVQQKPGQAPRGLIGGTKFLAPGTPARFSGSLLGGKAALTLSGVQPEDEAEYYCVLWYSNRWVFGGGTKLTVLHHHHHH

SEQ ID NO: 34 - protein, 728 aa, Artificial Sequence
  source: /note="Description of Artificial Sequence: Synthetic amino acid sequence of monomeric anti-CD33/CD3 Bi-Fc"
QVQLVQSGAEVKKPGESVKVSCKASGYTFTNYGMNWVKQAPGQGLEWMGWINTYTGEPTYADKFQGRVTMTTDTSTSTAYMEIRNLGGDDTAVYYCARWSWSDGYYVYFDYWGQGTSVTVSSGGGGSGGGGSGGGGSDIVMTQSPDSLTVSLGERTTINCKSSQSVLDSSTNKNSLAWYQQKPGQPPKLLLSWASTRESGIPDRFSGSGSGTDFTLTIDSPQPEDSATYYCQQSAHFPITFGQGTRLEIKSGGGGSEVQLVESGGGLVQPGGSLKLSCAASGFTFNKYAMNWVRQAPGKGLEWVARIRSKYNNYATYYADSVKDRFTISRDDSKNTAYLQMNNLKTEDTAVYYCVRHGNFGNSYISYWAYWGQGTLVTVSSGGGGSGGGGSGGGGSQTVVTQEPSLTVSPGGTVTLTCGSSTGAVTSGNYPNWVQQKPGQAPRGLIGGTKFLAPGTPARFSGSLLGGKAALTLSGVQPEDEAEYYCVLWYSNRWVFGGGTKLTVLAPELLGGPSVFLFPPKPKDTLMISRTPEVTCVVVDVSHEDPEVKFNWYVDGVEVHNAKTKPREEQYGSTYRVVSVLTVLHQDWLNGKEYKCKVSNKALPAPIEKTISKAKGQPREPQVTTLPPSREEMTKNQVSLTCLVKGFYPSDIAVEWESNGQPENNYDTTPPVLDSDGSFFLYSDLTVDKSRWQQGNVFSCSVMHEALHNHYTQKSLSLSPGKHHHHHH

SEQ ID NO: 35 - DNA, 1643 bp, Artificial Sequence
  source: /note="Description of Artificial Sequence: Synthetic nucleic acid sequence encoding SEQ ID NO:34"
caggtgcagctggtgcagtctggcgccgaagtgaagaaacctggagagtctgtcaaagtcagctgcaaggcctccggctacaccttcaccaactacggcatgaactgggtgaaacaggctccaggacagggactcgagtggatgggctggatcaacacctacaccggcgagcctacctacgccgacaagttccagggcagagtgaccatgaccaccgacacatctaccagcacagcttacatggaaatccggaacctgggcggcgacgacaccgccgtgtactactgcgcccggtggtcttggtccgacggctactacgtgtacttcgactactggggccagggcacctccgtgacagtgtccagcggagggggaggaagtggcggagggggctctggaggtggcggctccgacatcgtgatgacccagtcccccgactccctgaccgtgtccctgggcgagcggaccaccatcaactgcaagtcctcccagtccgtgctggactcctccaccaacaagaactccctggcctggtatcagcagaagcctggccagcctcctaagctgctgctctcttgggcttccaccagagagagcgggattcccgataggttctccggctctggctccggcaccgacttcaccctgaccatcgactcccctcagcctgaggactccgccacctactactgccagcagtccgcccacttccctatcaccttcggccagggaacccggctggaaatcaagtctggcggcggtggctctgaagtgcagctcgtggagagtggcggaggactggtgcagccaggcggctccctgaagctgtcttgcgccgccagcggcttcaccttcaataagtacgctatgaattgggtccggcaggcacctggaaaagggctcgaatgggtcgcaaggattaggtctaagtacaacaactacgccacctattacgccgactctgtgaaggaccggttcaccatctcccgggacgactctaagaacaccgcttacctgcagatgaacaacctgaaaaccgaggataccgctgtgtactattgtgtgcggcacggcaacttcggcaactcctacatctcctactgggcctattggggacagggcacactggtcaccgtgtcctctggcggtggaggatctggtggcggcggatctggcggcggaggttcccagaccgtggtcacccaggaaccttctctgaccgtcagtcccggcggaaccgtgaccctgacctgtggctcctctaccggcgctgtgacctccggcaactaccctaactgggtgcagcagaaacccggccaggctcccagaggactcatcggcggcaccaagtttctggcccctggcacccctgccagattctctggctccctgctgggcggcaaggctgctctgaccctgagcggagtccagccagaggacgaggccgagtactactgtgtgctgtggtactccaacagatgggtgttcggcggtggcaccaagctgaccgtgctggcacctgaactcctggggggaccgtcagtcttcctcttccccccaaaacccaaggacaccctcatgatctcccggacccctgaggtcacatgcgtggtggtggacgtgagccacgaagaccctgaggt

SEQ ID NO: 36 - protein, 12 aa, Artificial Sequence
  source: /note="Description of Artificial Sequence: Synthetic amino acid sequence of an insertion that prolongs half life"
GGCVFNMFNCGG

SEQ ID NO: 37 - protein, 12 aa, Artificial Sequence
  source: /note="Description of Artificial Sequence: Synthetic amino acid sequence of an insertion that prolongs half life"
GGCHLPFAVCGG

SEQ ID NO: 38 - protein, 12 aa, Artificial Sequence
  source: /note="Description of Artificial Sequence: Synthetic amino acid sequence of an insertion that prolongs half life"
GGCGHEYMWCGG

SEQ ID NO: 39 - protein, 12 aa, Artificial Sequence
  source: /note="Description of Artificial Sequence: Synthetic amino acid sequence of an insertion that prolongs half life"
GGCWPLQDYCGG

SEQ ID NO: 40 - protein, 12 aa, Artificial Sequence
  source: /note="Description of Artificial Sequence: Synthetic amino acid sequence of an insertion that prolongs half life"
GGCMQMNKWCGG

SEQ ID NO: 41 - protein, 12 aa, Artificial Sequence
  source: /note="Description of Artificial Sequence: Synthetic amino acid sequence of an insertion that prolongs half life"
GGCDGRTKYCGG

SEQ ID NO: 42 - protein, 12 aa, Artificial Sequence
  source: /note="Description of Artificial Sequence: Synthetic amino acid sequence of an insertion that prolongs half life"
GGCALYPTNCGG

SEQ ID NO: 43 - protein, 12 aa, Artificial Sequence
  source: /note="Description of Artificial Sequence: Synthetic amino acid sequence of an insertion that prolongs half life"
GGCGKHWHQCGG

SEQ ID NO: 44 - protein, 12 aa, Artificial Sequence
  source: /note="Description of Artificial Sequence: Synthetic amino acid sequence of an insertion that prolongs half life"
GGCHSFKHFCGG

SEQ ID NO: 45 - protein, 12 aa, Artificial Sequence
  source: /note="Description of Artificial Sequence: Synthetic amino acid sequence of an insertion that prolongs half life"
GGCQGMWTWCGG

SEQ ID NO: 46 - protein, 14 aa, Artificial Sequence
  source: /note="Description of Artificial Sequence: Synthetic amino acid sequence of an insertion that prolongs half life"
GGCAQQWHHEYCGG

SEQ ID NO: 47 - protein, 12 aa, Artificial Sequence
  source: /note="Description of Artificial Sequence: Synthetic amino acid sequence of an insertion that prolongs half life"
GGCERFHHACGG

SEQ ID NO: 48 - protein, 5 aa, Artificial Sequence
  source: /note="Description of Artificial Sequence: Synthetic amino acid sequence of a VH region CDR1 which is part of SEQ ID NO:7"
SYAMN

SEQ ID NO: 49 - protein, 19 aa, Artificial Sequence
  source: /note="Description of Artificial Sequence: Synthetic amino acid sequence of a VH region CDR2 which is part of SEQ ID NO:7"
RIRSKYNNYATYYADSVKG

SEQ ID NO: 50 - protein, 14 aa, Artificial Sequence
  source: /note="Description of Artificial Sequence: Synthetic amino acid sequence of a VH region CDR3 which is part of SEQ ID NO:7"
HGNFGNSYVSWWAY

SEQ ID NO: 51 - protein, 14 aa, Artificial Sequence
  source: /note="Description of Artificial Sequence: Synthetic amino acid sequence of a VL region CDR1 which is part of SEQ ID NO:8"
GSSTGAVTSGNYPN

SEQ ID NO: 52 - protein, 7 aa, Artificial Sequence
  source: /note="Description of Artificial Sequence: Synthetic amino acid sequence of a VL region CDR2 which is part of SEQ ID NO:8"
GTKFLAP

SEQ ID NO: 53 - protein, 9 aa, Artificial Sequence
  source: /note="Description of Artificial Sequence: Synthetic amino acid sequence of a VL region CDR3 which is part of SEQ ID NO:8"
VLWYSNRWV

SEQ ID NO: 54 - protein, 5 aa, Artificial Sequence
  source: /note="Description of Artificial Sequence: Synthetic amino acid sequence of a VH region CDR1 which is part of SEQ ID NO:29"
KYAMN

SEQ ID NO: 55 - protein, 19 aa, Artificial Sequence
  source: /note="Description of Artificial Sequence: Synthetic amino acid sequence of a VH region CDR2 which is part of SEQ ID NO:29"
RIRSKYNNYATYYADSVKD

SEQ ID NO: 56 - protein, 14 aa, Artificial Sequence
  source: /note="Description of Artificial Sequence: Synthetic amino acid sequence of a VH region CDR3 which is part of SEQ ID NO:29"
HGNFGNSYISYWAY

SEQ ID NO: 57 - protein, 14 aa, Artificial Sequence
  source: /note="Description of Artificial Sequence: Synthetic amino acid sequence of a VL region CDR1 which is part of SEQ ID NO:31"
GSSTGAVTSGNYPN

SEQ ID NO: 58 - protein, 7 aa, Artificial Sequence
  source: /note="Description of Artificial Sequence: Synthetic amino acid sequence of a VL region CDR2 which is part of SEQ ID NO:31"
GTKFLAP

SEQ ID NO: 59 - protein, 9 aa, Artificial Sequence
  source: /note="Description of Artificial Sequence: Synthetic amino acid sequence of a VL region CDR3 which is part of SEQ ID NO:31"
VLWYSNRWV

SEQ ID NO: 60 - protein, 5 aa, Artificial Sequence
  source: /note="Description of Artificial Sequence: Synthetic amino acid sequence of a VH CDR1 of SEQ ID NO:5"
DYFVN

SEQ ID NO: 61 - protein, 17 aa, Artificial Sequence
  source: /note="Description of Artificial Sequence: Synthetic amino acid sequence of a VH CDR2 of SEQ ID NO:5"
WIDPENDNSLYGPNFQD

SEQ ID NO: 62 - protein, 11 aa, Artificial Sequence
  source: /note="Description of Artificial Sequence: Synthetic amino acid sequence of a VH CDR3 of SEQ ID NO:5"
YYGSRGDAMDY

SEQ ID NO: 63 - protein, 11 aa, Artificial Sequence
  source: /note="Description of Artificial Sequence: Synthetic amino acid sequence of a VL CDR1 of SEQ ID NO:6"
RASQDISNYLN

SEQ ID NO: 64 - protein, 7 aa, Artificial Sequence
  source: /note="Description of Artificial Sequence: Synthetic amino acid sequence of a VL CDR2 of SEQ ID NO:6"
YTSRLHS

SEQ ID NO: 65 - protein, 9 aa, Artificial Sequence
  source: /note="Description of Artificial Sequence: Synthetic amino acid sequence of a VL CDR3 of SEQ ID NO:6"
QQGNTLPLT

SEQ ID NO: 66 - protein, 5 aa, Artificial Sequence
  source: /note="Description of Artificial Sequence: Synthetic amino acid sequence of a VH region CDR1 of SEQ ID NO:15"
SGAYY

SEQ ID NO: 67 - protein, 16 aa, Artificial Sequence
  source: /note="Description of Artificial Sequence: Synthetic amino acid sequence of a VH region CDR2 of SEQ ID NO:15"
YIYYSGSTYYNPSLKS

SEQ ID NO: 68 - protein, 8 aa, Artificial Sequence
  source: /note="Description of Artificial Sequence: Synthetic amino acid sequence of a VH region CDR2 of SEQ ID NO:15"
GSSSWFDY

SEQ ID NO: 69 - protein, 13 aa, Artificial Sequence
  source: /note="Description of Artificial Sequence: Synthetic amino acid sequence of a VL region CDR1 of SEQ ID NO:15"
SGSSSNIGNNAVN

SEQ ID NO: 70 - protein, 7 aa, Artificial Sequence
  source: /note="Description of Artificial Sequence: Synthetic amino acid sequence of a VL region CDR2 of SEQ ID NO:15"
YDDMLSS

SEQ ID NO: 71 - protein, 11 aa, Artificial Sequence
  source: /note="Description of Artificial Sequence: Synthetic amino acid sequence of a VL region CDR3 of SEQ ID NO:15"
AAWDDSLNGVV

SEQ ID NO: 72 - protein, 5 aa, Artificial Sequence
  source: /note="Description of Artificial Sequence: Synthetic amino acid sequence of a VH region CDR1 of SEQ ID NO:34"
NYGMN

SEQ ID NO: 73 - protein, 17 aa, Artificial Sequence
  source: /note="Description of Artificial Sequence: Synthetic amino acid sequence of a VH region CDR2 of SEQ ID NO:34"
WINTYTGEPTYADKFQG

SEQ ID NO: 74 - protein, 13 aa, Artificial Sequence
  source: /note="Description of Artificial Sequence: Synthetic amino acid sequence of a VH region CDR3 of SEQ ID NO:34"
WSWSDGYYVYFDY

SEQ ID NO: 75 - protein, 17 aa, Artificial Sequence
  source: /note="Description of Artificial Sequence: Synthetic amino acid sequence of a VL region CDR1 of SEQ ID NO:34"
KSSQSVLDSSTNKNSLA

SEQ ID NO: 76 - protein, 7 aa, Artificial Sequence
  source: /note="Description of Artificial Sequence: Synthetic amino acid sequence of a VL region CDR2 of SEQ ID NO:34"
WASTRES

SEQ ID NO: 77 - protein, 9 aa, Artificial Sequence
  source: /note="Description of Artificial Sequence: Synthetic amino acid sequence of a VL region CDR3 of SEQ ID NO:34"
QQSAHFPIT

SEQ ID NO: 78 - protein, 508 aa, Artificial Sequence
  source: /note="Description of Artificial Sequence: Synthetic amino acid sequence of an anti-Mec/CD3-epsilon single chain bispecific (P137424.7)"
VLTQTPSPVSAAVGGTVTINCQSSPSLIYDSRLAWYQQKPGQPPKLLIYKASTLASGVPSRFSGSGSGTQFTLTISDVQSDDAATYYCQSHDTNPGSSTYGAPFGGGTEVVVQGGGGSGGGGSSGGGSEVQLMESGGGLVKPEGSLTLTCKVSGFSFSTSAISWVRQAPGKRPEWIAGIYNGGGSTYYASWVNGRFSISRSTSLNTVTLQMTRLTAADTATYFCARWIRIHYSFDLWGPGTLVTVSSSGGGGSEVQLVESGGGLVQPGGSLKLSCAASGFTFNKYAMNWVRQAPGKGLEWVARIRSKYNNYATYYADSVKDRFTISRDDSKNTAYLQMNNLKTEDTAVYYCVRHGNFGNSYISYWAYWGQGTLVTVSSGGGGSGGGGSGGGGSQTVVTQEPSLTVSPGGTVTLTCGSSTGAVTSGNYPNWVQQKPGQAPRGLIGGTKFLAPGTPARFSGSLLGGKAALTLSGVQPEDEAEYYCVLWYSNRWVFGGGTKLTVLHHHHHH

SEQ ID NO: 79 - DNA, 1527 bp, Artificial Sequence
  source: /note="Description of Artificial Sequence: Synthetic Polynucleotide sequence encoding the amino acid sequence of the anti-Mec/CD3-epsilon single chain bispecific (P137424.7)"
gtcctcactcagaccccttctccggtctccgcggccgtcggcggaactgtcactatcaattgccagagttccccaagtctgatctatgacagtagattagcctggtatcagcaaaaaccagggcaaccacctaagctcctgatctataaagcatccactttggccagtggggtcccatcaaggttcagcggcagtggatctgggacacagttcactctcacaatcagcgacgtccagtctgacgatgccgcaacttattactgtcaaagtcatgacactaatcctgggtctagtacttatggcgccccattcggaggaggcactgaagtcgtagtccagggtggtggtggttctggcggcggcggctccagtggtggtggttctgaggtgcagctgatggagtctgggggaggcttggtaaagcccgaggggtccctgaccctcacctgcaaggtctctggattctccttttcaacgagtgccattagctgggtccgccaggctccagggaagagaccagagtggatcgccgggatttataacggaggtggtagcacatactacgcatcctgggtgaacggccggttcagcatctccagatccacgtccttgaacacggtgacgctgcaaatgaccagactgacggccgctgacacggccacatatttctgtgcgagatggattcggatccattattccttcgacctgtggggacctggcacgttggtcaccgtctcctcatccggaggtggtggctccgaggtgcagctggtcgagtctggaggaggattggtgcagcctggagggtcattgaaactctcatgtgcagcctctggattcaccttcaataagtacgccatgaactgggtccgccaggctccaggaaagggtttggaatgggttgctcgcataagaagtaaatataataattatgcaacatattatgccgattcagtgaaagacaggttcaccatctccagagatgattcaaaaaacactgcctatctacaaatgaacaacttgaaaactgaggacactgccgtgtactactgtgtgagacatgggaacttcggtaatagctacatatcctactgggcttactggggccaagggactctggtcaccgtctcctcaggtggtggtggttctggcggcggcggctccggtggtggtggttctcagactgttgtgactcaggaaccttcactcaccgtatcacctggtggaacagtcacactcacttgtggctcctcgactggggctgttacatctggcaactacccaaactgggtccaacaaaaaccaggtcaggcaccccgtggtctaataggtgggactaagttcctcgcccccggtactcctgccagattctcaggctccctgcttggaggcaaggctgccctcaccctctcaggggtacagccagaggatgaggcagaatattactgtgttctatggtacagcaaccgctgggtgttcggtggaggaaccaaactgactgtcctacatcatcaccatcatcattag

SEQ ID NO: 80 - protein, 743 aa, Artificial Sequence
  source: /note="Description of Artificial Sequence: Synthetic amino acid sequence of the first polypeptide chain of a heterodimeric anti-CD33/CD3-epsilon Bi-Fc aCD33(AMG330) -scFv-aCD3(I2C)-scFv-Fc(L234A, L235A, E356K, D399K (PL-31769)"
QVQLVQSGAEVKKPGESVKVSCKASGYTFTNYGMNWVKQAPGQGLEWMGWINTYTGEPTYADKFQGRVTMTTDTSTSTAYMEIRNLGGDDTAVYYCARWSWSDGYYVYFDYWGQGTSVTVSSGGGGSGGGGSGGGGSDIVMTQSPDSLTVSLGERTTINCKSSQSVLDSSTNKNSLAWYQQKPGQPPKLLLSWASTRESGIPDRFSGSGSGTDFTLTIDSPQPEDSATYYCQQSAHFPITFGQGTRLEIKSGGGGSEVQLVESGGGLVQPGGSLKLSCAASGFTFNKYAMNWVRQAPGKGLEWVARIRSKYNNYATYYADSVKDRFTISRDDSKNTAYLQMNNLKTEDTAVYYCVRHGNFGNSYISYWAYWGQGTLVTVSSGGGGSGGGGSGGGGSQTVVTQEPSLTVSPGGTVTLTCGSSTGAVTSGNYPNWVQQKPGQAPRGLIGGTKFLAPGTPARFSGSLLGGKAALTLSGVQPEDEAEYYCVLWYSNRWVFGGGTKLTVLEPKSSDKTHTCPPCPAPEAAGGPSVFLFPPKPKDTLMISRTPEVTCVVVDVSHEDPEVKFNWYVDGVEVHNAKTKPREEQYNSTYRVVSVLTVLHQDWLNGKEYKCKVSNKALPAPIEKTISKAKGQPREPQVYTLPPSRKEMTKNQVSLTCLVKGFYPSDIAVEWESNGQPENNYKTTPPVLKSDGSFFLYSKLTVDKSRWQQGNVFSCSVMHEALHNHYTQKSLSLSPGKHHHHHH

SEQ ID NO: 81 - DNA, 2232 bp, Artificial Sequence
  source: /note="Description of Artificial Sequence: Synthetic nucleic acid sequence encoding SEQ ID NO:80"
caggtgcagctggtgcagtctggcgccgaagtgaagaaacctggagagtctgtcaaagtcagctgcaaggcctccggctacaccttcaccaactacggcatgaactgggtgaaacaggctccaggacagggactcgagtggatgggctggatcaacacctacaccggcgagcctacctacgccgacaagttccagggcagagtgaccatgaccaccgacacatctaccagcacagcttacatggaaatccggaacctgggcggcgacgacaccgccgtgtactactgcgcccggtggtcttggtccgacggctactacgtgtacttcgactactggggccagggcacctccgtgacagtgtccagcggagggggaggaagtggcggagggggctctggaggtggcggctccgacatcgtgatgacccagtcccccgactccctgaccgtgtccctgggcgagcggaccaccatcaactgcaagtcctcccagtccgtgctggactcctccaccaacaagaactccctggcctggtatcagcagaagcctggccagcctcctaagctgctgctctcttgggcttccaccagagagagcgggattcccgataggttctccggctctggctccggcaccgacttcaccctgaccatcgactcccctcagcctgaggactccgccacctactactgccagcagtccgcccacttccctatcaccttcggccagggaacccggctggaaatcaagtctggcggcggtggctctgaagtgcagctcgtggagagtggcggaggactggtgcagccaggcggctccctgaagctgtcttgcgccgccagcggcttcaccttcaataagtacgctatgaattgggtccggcaggcacctggaaaagggctcgaatgggtcgcaaggattaggtctaagtacaacaactacgccacctattacgccgactctgtgaaggaccggttcaccatctcccgggacgactctaagaacaccgcttacctgcagatgaacaacctgaaaaccgaggataccgctgtgtactattgtgtgcggcacggcaacttcggcaactcctacatctcctactgggcctattggggacagggcacactggtcaccgtgtcctctggcggtggaggatctggtggcggcggatctggcggcggaggttcccagaccgtggtcacccaggaaccttctctgaccgtcagtcccggcggaaccgtgaccctgacctgtggctcctctaccggcgctgtgacctccggcaactaccctaactgggtgcagcagaaacccggccaggctcccagaggactcatcggcggcaccaagtttctggcccctggcacccctgccagattctctggctccctgctgggcggcaaggctgctctgaccctgagcggagtccagccagaggacgaggccgagtactactgtgtgctgtggtactccaacagatgggtgttcggcggtggcaccaagctgaccgtgctggagcccaaatcttctgacaaaactcacacatgccccccgtgcccagcacctgaagcagctgggggaccgtcagtcttcctcttccccccaaaacccaaggacaccctcatgatctcccggacccctgaggtcacatgcgtggtggtggacgtgagccacgaagaccctgaggtcaagttcaactggtacgtggacggcgtggaggtgcataatgccaagacaaagccgcgagaggagcagtacaacagcacgtaccgtgtggtcagcgtcctcaccgtcctgcaccaggactggctgaatggcaaggagtacaagtgcaaggtctccaacaaagccctcccagcccccatcgagaaaaccatctccaaagccaaagggcagccccgagaaccacaggtgtacaccctgcccccatcccggaaggagatgaccaagaaccaggtcagcctgacctgcctggtcaaaggcttctatcccagcgacatcgccgtggagtgggagagcaatgggcagccggagaacaactacaagaccacgcctcccgtgctgaagtccgacggctccttcttcctctatagcaagctcaccgtggacaagagcaggtggcagcaggggaacgtcttctcatgctccgtgatgcatgaggctctgcacaaccactacacgcagaagagcctctccctgtctccgggtaaacatcatcatcatcatcattaa

SEQ ID NO: 82 - protein, 243 aa, Artificial Sequence; identical to SEQ ID NO: 12
  source: /note="Description of Artificial Sequence: Synthetic amino acid sequence of an Fc polypeptide chain dummyFc-AADD"

SEQ ID NO: 83 - DNA, 729 bp, Artificial Sequence; identical to SEQ ID NO: 13
  source: /note="Description of Artificial Sequence: Synthetic nucleic acid sequence encoding SEQ ID NO:82"

SEQ ID NO: 84 - protein, 728 aa, Artificial Sequence
  source: /note="Description of Artificial Sequence: Synthetic amino acid sequence of a monomeric anti-CD33/CD3 Bi-Fc having the wild type sequence at residue N297 in the Fc portion of the molecule aCD33(AMF330)scFv-aCD3(I2C)scFv-Fc-mono"
QVQLVQSGAEVKKPGESVKVSCKASGYTFTNYGMNWVKQAPGQGLEWMGWINTYTGEPTYADKFQGRVTMTTDTSTSTAYMEIRNLGGDDTAVYYCARWSWSDGYYVYFDYWGQGTSVTVSSGGGGSGGGGSGGGGSDIVMTQSPDSLTVSLGERTTINCKSSQSVLDSSTNKNSLAWYQQKPGQPPKLLLSWASTRESGIPDRFSGSGSGTDFTLTIDSPQPEDSATYYCQQSAHFPITFGQGTRLEIKSGGGGSEVQLVESGGGLVQPGGSLKLSCAASGFTFNKYAMNWVRQAPGKGLEWVARIRSKYNNYATYYADSVKDRFTISRDDSKNTAYLQMNNLKTEDTAVYYCVRHGNFGNSYISYWAYWGQGTLVTVSSGGGGSGGGGSGGGGSQTVVTQEPSLTVSPGGTVTLTCGSSTGAVTSGNYPNWVQQKPGQAPRGLIGGTKFLAPGTPARFSGSLLGGKAALTLSGVQPEDEAEYYCVLWYSNRWVFGGGTKLTVLAPELLGGPSVFLFPPKPKDTLMISRTPEVTCVVVDVSHEDPEVKFNWYVDGVEVHNAKTKPREEQYNSTYRVVSVLTVLHQDWLNGKEYKCKVSNKALPAPIEKTISKAKGQPREPQVTTLPPSREEMTKNQVSLTCLVKGFYPSDIAVEWESNGQPENNYDTTPPVLDSDGSFFLYSDLTVDKSRWQQGNVFSCSVMHEALHNHYTQKSLSLSPGKHHHHHH

SEQ ID NO: 85 - DNA, 2187 bp, Artificial Sequence
  source: /note="Description of Artificial Sequence: Synthetic nucleic acid sequence encoding SEQ ID NO:84"
caggtgcagctggtgcagtctggcgccgaagtgaagaaacctggagagtctgtcaaagtcagctgcaaggcctccggctacaccttcaccaactacggcatgaactgggtgaaacaggctccaggacagggactcgagtggatgggctggatcaacacctacaccggcgagcctacctacgccgacaagttccagggcagagtgaccatgaccaccgacacatctaccagcacagcttacatggaaatccggaacctgggcggcgacgacaccgccgtgtactactgcgcccggtggtcttggtccgacggctactacgtgtacttcgactactggggccagggcacctccgtgacagtgtccagcggagggggaggaagtggcggagggggctctggaggtggcggctccgacatcgtgatgacccagtcccccgactccctgaccgtgtccctgggcgagcggaccaccatcaactgcaagtcctcccagtccgtgctggactcctccaccaacaagaactccctggcctggtatcagcagaagcctggccagcctcctaagctgctgctctcttgggcttccaccagagagagcgggattcccgataggttctccggctctggctccggcaccgacttcaccctgaccatcgactcccctcagcctgaggactccgccacctactactgccagcagtccgcccacttccctatcaccttcggccagggaacccggctggaaatcaagtctggcggcggtggctctgaagtgcagctcgtggagagtggcggaggactggtgcagccaggcggctccctgaagctgtcttgcgccgccagcggcttcaccttcaataagtacgctatgaattgggtccggcaggcacctggaaaagggctcgaatgggtcgcaaggattaggtctaagtacaacaactacgccacctattacgccgactctgtgaaggaccggttcaccatctcccgggacgactctaagaacaccgcttacctgcagatgaacaacctgaaaaccgaggataccgctgtgtactattgtgtgcggcacggcaacttcggcaactcctacatctcctactgggcctattggggacagggcacactggtcaccgtgtcctctggcggtggaggatctggtggcggcggatctggcggcggaggttcccagaccgtggtcacccaggaaccttctctgaccgtcagtcccggcggaaccgtgaccctgacctgtggctcctctaccggcgctgtgacctccggcaactaccctaactgggtgcagcagaaacccggccaggctcccagaggactcatcggcggcaccaagtttctggcccctggcacccctgccagattctctggctccctgctgggcggcaaggctgctctgaccctgagcggagtccagccagaggacgaggccgagtactactgtgtgctgtggtactccaacagatgggtgttcggcggtggcaccaagctgaccgtgctggcacctgaactcctggggggaccgtcagtcttcctcttccccccaaaacccaaggacaccctcatgatctcccggacccctgaggtcacatgcgtggtggtggacgtgagccacgaagaccctgaggtcaagttcaactggtacgtggacggcgtggaggtgcataatgccaagacaaagccgcgggaggagcagtacaacagcacgtaccgtgtggtcagcgtcctcaccgtcctgcaccaggactggctgaatggcaaggagtacaagtgcaaggtctccaacaaagccctcccagcccccatcgagaaaaccatctccaaagccaaagggcagccccgagaaccacaggtgactaccctgcccccatcccgggaggagatgaccaagaaccaggtcagcctgacctgcctggtcaaaggcttctatcccagcgacatcgccgtggagtgggagagcaatgggcagccggagaacaactacgacaccacgcctcccgtgctggactccgacggctccttcttcctctatagcgacctcaccgtggacaagagcaggtggcagcaggggaacgtcttctcatgctccgtgatgcatgaggctctgcacaaccactacacgcagaagagcctctccctgtctccgggtaaacatcatcatcatcatcattga

SEQ ID NO: 86 - protein, 736 aa, Artificial Sequence
  source: /note="Description of Artificial Sequence: Synthetic amino acid sequence of anti-FOLR1/CD3-epsilon Bi-Fc (PL-30058) ahuFolateR-1(5G1)-scFv-ahuCD3(I2C)scFv-FcAAKK"
QVQLQESGPGLVKPSQTLSLTCTVSGGSISSGAYYWTWIRQHPGKGLEWIGYIYYSGSTYYNPSLKSRVSISIDTSKNQFSLKLSSVTAADTAVYYCARGSSSWFDYWGQGTLVTVSSGGGGSGGGGSGGGGSQSVLTQPPSVSEAPRQRVTISCSGSSSNIGNNAVNWYQQLPGKAPKLLIYYDDMLSSGVSDRFSGSKSGTSASLAISGLQSEDEADYYCAAWDDSLNGVVFGGGTKLTVLSGGGGSEVQLVESGGGLVQPGGSLKLSCAASGFTFNKYAMNWVRQAPGKGLEWVARIRSKYNNYATYYADSVKDRFTISRDDSKNTAYLQMNNLKTEDTAVYYCVRHGNFGNSYISYWAYWGQGTLVTVSSGGGGSGGGGSGGGGSQTVVTQEPSLTVSPGGTVTLTCGSSTGAVTSGNYPNWVQQKPGQAPRGLIGGTKFLAPGTPARFSGSLLGGKAALTLSGVQPEDEAEYYCVLWYSNRWVFGGGTKLTVLEPKSSDKTHTCPPCPAPEAAGGPSVFLFPPKPKDTLMISRTPEVTCVVVDVSHEDPEVKFNWYVDGVEVHNAKTKPREEQYNSTYRVVSVLTVLHQDWLNGKEYKCKVSNKALPAPIEKTISKAKGQPREPQVYTLPPSRKEMTKNQVSLTCLVKGFYPSDIAVEWESNGQPENNYKTTPPVLKSDGSFFLYSKLTVDKSRWQQGNVFSCSVMHEALHNHYTQKSLSLSPGKHHHHHH

SEQ ID NO: 87 - DNA, 2211 bp, Artificial Sequence
  source: /note="Description of Artificial Sequence: Synthetic nucleic acid sequence encoding SEQ ID NO:86"
caggtgcagctgcaggagtcgggcccaggactggtgaagccttcacagaccctgtccctcacctgcactgtctctggtggctccatcagcagtggtgcttactactggacctggatccgccagcacccagggaagggcctggagtggattgggtacatctattacagtgggagcacctactacaacccgtccctcaagagtcgagttagcatatcaatagacacgtctaagaaccagttctccctgaagctgagctctgtgactgccgcggacacggccgtgtattactgtgcgcgaggcagcagcagctggttcgactactggggccagggaaccctggtcaccgtctcctcaggaggcggcggttcaggcggaggtggctctggcggtggcggaagtcagtctgtgctgactcagccaccctcggtgtctgaagcccccaggcagagggtcaccatctcctgttctggaagcagctccaacatcggaaataatgctgtaaactggtaccagcagctcccaggaaaggctcccaaactcctcatctattatgatgatatgttgtcttcaggggtctcggaccgattttctggctccaagtctggcacctcagcctccctggccatcagtgggctccagtctgaggatgaggctgattattactgtgcagcatgggatgacagcctgaatggtgtggtattcggcggagggaccaagctgaccgtcctatccggaggtggtggatccgaagtgcagctcgtggagagtggcggaggactggtgcagccaggcggctccctgaagctgtcttgcgccgccagcggcttcaccttcaataagtacgctatgaattgggtccggcaggcacctggaaaagggctcgaatgggtcgcaaggattaggtctaagtacaacaactacgccacctattacgccgactctgtgaaggaccggttcaccatctcccgggacgactctaagaacaccgcttacctgcagatgaacaacctgaaaaccgaggataccgctgtgtactattgtgtgcggcacggcaacttcggcaactcctacatctcctactgggcctattggggacagggcacactggtcaccgtgtcctctggcggtggaggatctggtggcggcggatctggcggcggaggttcccagaccgtggtcacccaggaaccttctctgaccgtcagtcccggcggaaccgtgaccctgacctgtggctcctctaccggcgctgtgacctccggcaactaccctaactgggtgcagcagaaacccggccaggctcccagaggactcatcggcggcaccaagtttctggcccctggcacccctgccagattctctggctccctgctgggcggcaaggctgctctgaccctgagcggagtccagccagaggacgaggccgagtactactgtgtgctgtggtactccaacagatgggtgttcggcggtggcaccaagctgaccgtgctggagcccaaatcttctgacaaaactcacacatgccccccgtgcccagcacctgaagcagctgggggaccgtcagtcttcctcttccccccaaaacccaaggacaccctcatgatctcccggacccctgaggtcacatgcgtggtggtggacgtgagccacgaagaccctgaggtcaagttcaactggtacgtggacggcgtggaggtgcataatgccaagacaaagccgcgagaggagcagtacaacagcacgtaccgtgtggtcagcgtcctcaccgtcctgcaccaggactggctgaatggcaaggagtacaagtgcaaggtctccaacaaagccctcccagcccccatcgagaaaaccatctccaaagccaaagggcagccccgagaaccacaggtgtacaccctgcccccatcccggaaggagatgaccaagaaccaggtcagcctgacctgcctggtcaaaggcttctatcccagcgacatcgccgtggagtgggagagcaatgggcagccggagaacaactacaagaccacgcctcccgtgctgaagtccgacggctccttcttcctctatagcaagctcaccgtggacaagagcaggtggcagcaggggaacgtcttctcatgctccgtgatgcatgaggctctgcacaaccactacacgcagaagagcctctccctgtctccgggtaaacatcaccaccaccatcactga

SEQ ID NO: 88 - protein, 243 aa, Artificial Sequence; identical to SEQ ID NO: 12
  source: /note="Description of Artificial Sequence: Synthetic amino acid sequence encoding an Fc polypeptide chain"

SEQ ID NO: 89 - DNA, 729 bp, Artificial Sequence; identical to SEQ ID NO: 13
  source: /note="Description of Artificial Sequence: Synthetic nucleic acid sequence encoding SEQ ID NO:88"

SEQ ID NO: 90 - protein, 504 aa, Artificial Sequence
  source: /note="Description of Artificial Sequence: Synthetic Amino acid sequence of a single chain anti-FOLR1/CD3-epsilon Bispecific PL-30055 aFOLR1(5G1)scFv-aCD3(I2C)scFv"
QVQLQESGPGLVKPSQTLSLTCTVSGGSISSGAYYWTWIRQHPGKGLEWIGYIYYSGSTYYNPSLKSRVSISIDTSKNQFSLKLSSVTAADTAVYYCARGSSSWFDYWGQGTLVTVSSGGGGSGGGGSGGGGSQSVLTQPPSVSEAPRQRVTISCSGSSSNIGNNAVNWYQQLPGKAPKLLIYYDDMLSSGVSDRFSGSKSGTSASLAISGLQSEDEADYYCAAWDDSLNGVVFGGGTKLTVLSGGGGSEVQLVESGGGLVQPGGSLKLSCAASGFTFNKYAMNWVRQAPGKGLEWVARIRSKYNNYATYYADSVKDRFTISRDDSKNTAYLQMNNLKTEDTAVYYCVRHGNFGNSYISYWAYWGQGTLVTVSSGGGGSGGGGSGGGGSQTVVTQEPSLTVSPGGTVTLTCGSSTGAVTSGNYPNWVQQKPGQAPRGLIGGTKFLAPGTPARFSGSLLGGKAALTLSGVQPEDEAEYYCVLWYSNRWVFGGGTKLTVLHHHHHH

SEQ ID NO: 91 - DNA, 1515 bp, Artificial Sequence
  source: /note="Description of Artificial Sequence: Synthetic nucleic acid sequence encoding SEQ ID NO:90"
caggtgcagctgcaggagtcgggcccaggactggtgaagccttcacagaccctgtccctcacctgcactgtctctggtggctccatcagcagtggtgcttactactggacctggatccgccagcacccagggaagggcctggagtggattgggtacatctattacagtgggagcacctactacaacccgtccctcaagagtcgagttagcatatcaatagacacgtctaagaaccagttctccctgaagctgagctctgtgactgccgcggacacggccgtgtattactgtgcgcgaggcagcagcagctggttcgactactggggccagggaaccctggtcaccgtctcctcaggaggcggcggttcaggcggaggtggctctggcggtggcggaagtcagtctgtgctgactcagccaccctcggtgtctgaagcccccaggcagagggtcaccatctcctgttctggaagcagctccaacatcggaaataatgctgtaaactggtaccagcagctcccaggaaaggctcccaaactcctcatctattatgatgatatgttgtcttcaggggtctcggaccgattttctggctccaagtctggcacctcagcctccctggccatcagtgggctccagtctgaggatgaggctgattattactgtgcagcatgggatgacagcctgaatggtgtggtattcggcggagggaccaagctgaccgtcctatccggaggtggtggatccgaagtgcagctcgtggagagtggcggaggactggtgcagccaggcggctccctgaagctgtcttgcgccgccagcggcttcaccttcaataagtacgctatgaattgggtccggcaggcacctggaaaagggctcgaatgggtcgcaaggattaggtctaagtacaacaactacgccacctattacgccgactctgtgaaggaccggttcaccatctcccgggacgactctaagaacaccgcttacctgcagatgaacaacctgaaaaccgaggataccgctgtgtactattgtgtgcggcacggcaacttcggcaactcctacatctcctactgggcctattggggacagggcacactggtcaccgtgtcctctggcggtggaggatctggtggcggcggatctggcggcggaggttcccagaccgtggtcacccaggaaccttctctgaccgtcagtcccggcggaaccgtgaccctgacctgtggctcctctaccggcgctgtgacctccggcaactaccctaactgggtgcagcagaaacccggccaggctcccagaggactcatcggcggcaccaagtttctggcccctggcacccctgccagattctctggctccctgctgggcggcaaggctgctctgaccctgagcggagtccagccagaggacgaggccgagtactactgtgtgctgtggtactccaacagatgggtgttcggcggtggcaccaagctgaccgtgctgcatcaccaccaccatcactga

SEQ ID NO: 92 - protein, 6 aa, Artificial Sequence
  source: /note="Description of Artificial Sequence: Synthetic 6xHis tag"
HHHHHH